European Patent Application EP 4 375 298 A1, published May 29, 2024. Title: PHARMACEUTICAL COMPOSITION OF ANTI-ANGPTL3 ANTIBODY OR ANTIGEN BINDING FRAGMENT THEREOF AND ITS APPLICATION. Applicant: JIANGSU HENGRUI PHARMACEUTICALS CO., LTD. Application CN PCT/CN2022/106993, filed July 21, 2022. The sequence listing filed with the application follows.

SEQUENCE LISTING (22 sequences)

SEQ ID NO: 1 - protein, 473 aa, synthetic construct
MEFGLSWLFLVAILKGVQCSRIDQDNSSFDSLSPEPKSRFAMLDDVKILANGLLQLGHGLKDFVHKTKGQINDIFQKLNIFDQSFYDLSLQTSEIKEEEKELRRTTYKLQVKNEEVKNMSLELNSKLESLLEEKILLQQKVKYLEEQLTNLIQNQPETPEHPEVTSLKTFVEKQDNSIKDLLQTVEDQYKQLNQQHSQIKEIENQLRRTSIQEPTEISLSSKPRAPRTTPFLQLNEIRNVKHDGIPAECTTIYNRGEHTSGMYAIRPSNSQVFHVYCDVISGSPWTLIQHRIDGSQNFNETWENYKYGFGRLDGEFWLGLEKIYSIVKQSNYVLRIELEDWKDNKHYIEYSFYLGNHETNYTLHLVAITGNVPNAIPENKDLVFSTWDHKAKGHFNCPEGYSGGWWWHDECGENNLNGKYNKPRAKSKPERRRGLSWKSQNGRLYSIKSTKMLIHPTDSESFEHHHHHHHHHH

SEQ ID NO: 2 - protein, 190 aa, synthetic construct
MEFGLSWLFLVAILKGVQCSRIDQDNSSFDSLSPEPKSRFAMLDDVKILANGLLQLGHGLKDFVHKTKGQINDIFQKLNIFDQSFYDLSLQTSEIKEEEKELRRTTYKLQVKNEEVKNMSLELNSKLESLLEEKILLQQKVKYLEEQLTNLIQNQPETPEHPEVTSLKTFVEKGSSDYKDDDDKHHHHHH

SEQ ID NO: 3 - protein, 406 aa, synthetic construct
MEFGLSWLFLVAILKGVQCSRIDQDNSSFDSLSPEPKSRFAMLDDVKILANGLLQLGHGLKDFVHKTKGQINDIFQKLNIFDQSFYDLSLQTSEIKEEEKELRRTTYKLQVKNEEVKNMSLELNSKLESLLEEKILLQQKVKYLEEQLTNLIQNQPETPEHPEVTSLKTFVEKEPRGPTIKPCPPCKCPAPNLLGGPSVFIFPPKIKDVLMISLSPIVTCVVVDVSEDDPDVQISWFVNNVEVHTAQTQTHREDYNSTLRVVSALPIQHQDWMSGKEFKCKVNNKDLPAPIERTISKPKGSVRAPQVYVLPPPEEEMTKKQVTLTCMVTDFMPEDIYVEWTNNGKTELNYKNTEPVLDSDGSYFMYSKLRVEKKNWVERNSYSCSVVHEGLHNHHTTKSFSRTPGK

SEQ ID NO: 4 - protein, 456 aa, synthetic construct
MEFGLSWLFLVAILKGVQCSRIDQDNSSFDSLSPEPKSRFAMLDDVKILANGLLQLGHGLKDFVHKTKGQINDIFQKLNIFDQSFYDLSLQTSEIKEEEKELRRTTYKLQVKNEEVKNMSLELNSKLESLLEEKILLQQKVKYLEEQLTNLIQNQPETPEHPEVTSLKTFVEKQDNSIKDLLQTVEDQYKQLNQQHSQIKEIENQLRRTSIQEPTEISLSSKPEPRGPTIKPCPPCKCPAPNLLGGPSVFIFPPKIKDVLMISLSPIVTCVVVDVSEDDPDVQISWFVNNVEVHTAQTQTHREDYNSTLRVVSALPIQHQDWMSGKEFKCKVNNKDLPAPIERTISKPKGSVRAPQVYVLPPPEEEMTKKQVTLTCMVTDFMPEDIYVEWTNNGKTELNYKNTEPVLDSDGSYFMYSKLRVEKKNWVERNSYSCSVVHEGLHNHHTTKSFSRTPGK

SEQ ID NO: 5 - protein, 468 aa, synthetic construct
MEFGLSWLFLVAILKGVQCSRVDPDLSSFDSAPSEPKSRFAMLDDVKILANGLLQLGHGLKDFVHKTKGQINDIFQKLNIFDQSFYDLSLRTNEIKEEEKELRRTTSTLQVKNEEVKNMSVELNSKLESLLEEKTALQHKVRALEEQLTNLILSPAGAQEHPEVTSLKSFVEQQDNSIRELLQSVEEQYKQLSQQHMQIKEIEKQLRKTGIQEPSENSLSSKSRAPRTTPPLQLNETENTEQDDLPADCSAVYNRGEHTSGVYTIKPRNSQGFNVYCDTQSGSPWTLIQHRKDGSQDFNETWENYEKGFGRLDGEFWLGLEKIYAIVQQSNYILRLELQDWKDSKHYVEYSFHLGSHETNYTLHVAEIAGNIPGALPEHTDLMFSTWNHRAKGQLYCPESYSGGWWWNDICGENNLNGKYNKPRTKSRPERRRGIYWRPQSRKLYAIKSSKMMLQPTTHHHHHHHHHH

SEQ ID NO: 6 - protein, 456 aa, synthetic construct
MEFGLSWLFLVAILKGVQCSRVDPDLSSFDSAPSEPKSRFAMLDDVKILANGLLQLGHGLKDFVHKTKGQINDIFQKLNIFDQSFYDLSLRTNEIKEEEKELRRTTSTLQVKNEEVKNMSVELNSKLESLLEEKTALQHKVRALEEQLTNLILSPAGAQEHPEVTSLKSFVEQQDNSIRELLQSVEEQYKQLSQQHMQIKEIEKQLRKTGIQEPSENSLSSKSEPRGPTIKPCPPCKCPAPNLLGGPSVFIFPPKIKDVLMISLSPIVTCVVVDVSEDDPDVQISWFVNNVEVHTAQTQTHREDYNSTLRVVSALPIQHQDWMSGKEFKCKVNNKDLPAPIERTISKPKGSVRAPQVYVLPPPEEEMTKKQVTLTCMVTDFMPEDIYVEWTNNGKTELNYKNTEPVLDSDGSYFMYSKLRVEKKNWVERNSYSCSVVHEGLHNHHTTKSFSRTPGK

SEQ ID NO: 7 - protein, 473 aa, synthetic construct
MEFGLSWLFLVAILKGVQCSRIDQDNSSFDSVSPEPKSRFAMLDDVKILANGLLQLGHGLKDFVHKTKGQINDIFQKLNIFDQSFYDLSLQTSEIKEEEKELRRTTYKLQVKNEEVKNMSLELNSKLESLLEEKILLQQKVKYLEEQLTNLIQNQPATPEHPEVTSLKSFVEKQDNSIKDLLQTVEEQYKQLNQQHSQIKEIENQLRMTNIQEPTEISLSSKPRAPRTTPFLQLNEIRNVKHDGIPADCTTIYNRGEHISGTYAIRPSNSQVFHVYCDVVSGSPWTLIQHRIDGSQNFNETWENYKYGFGRLDGEFWLGLEKIYSIVKQSNYVLRIELEDWKDNKHYIEYSFYLGNHETNYTLHVVKITGNVPNAIPENKDLVFSTWDHKAKGHFSCPESYSGGWWWHDECGENNLNGKYNKPRTKSKPERRRGLSWKSQNGRLYSIKSTKMLIHPTDSESFEHHHHHHHHHH

SEQ ID NO: 8 - protein, 468 aa, synthetic construct
MEFGLSWLFLVAILKGVQCSRVDPDLSPFDSVPSEPKSRFAMLDDVKILANGLLQLGHGLKDFVHKTKGQINDIFQKLNIFDQCFYDLSLQTNEIKEEEKELRRTTSKLQVKNEEVKNMSLELNSKLESLLEEKMALQHRVRALEEQLTSLVQNPPGAREHPEVTSLKSFVEQQDNSIRELLQSVEEQYKQLSQQHIQIKEIENQLRKTGIQEPTENSLYSKPRAPRTTPPLHLKEAKNIEQDDLPADCSAIYNRGEHTSGVYTIRPSSSQVFNVYCDTQSGTPRTLIQHRKDGSQNFNQTWENYEKGFGRLDGEFWLGLEKIYAIVKQSNYILRLELQDWKDSKHYAEYSFHLGNHETNYTLHVAEIAANIPEALPEHRDLMFSTWDHRAKGQLYCPESYSGGWWFSDMCGENNLNGKYNKPRAKSKPERRRGISWRPRGGKLYSIKSSKMMLQPTTHHHHHHHHHH

SEQ ID NO: 9 - protein, 124 aa, synthetic construct
QVQLVQSGAEVKKPGASVKVSCKASGYTFTSYDINWVRQAPGQGLEWVGLINPRDDSTSYAQKFQGRVTMTRDTSTSTMYMELSSLRSEDTAVYFCARDLGSIREVLYYGMDVWGQGTTVTVSS

SEQ ID NO: 10 - protein, 112 aa, synthetic construct
DVVMTQSPLSLPVTPGEPASISCRSSQSLLHSNGYTYLDWYLQKPGQSPQLLIYLGSNRASGVPDRFSGSGSGTDFTLKISRVEAEDVGVYYCMQALQTPLTFGQGTRLEIK

SEQ ID NO: 11 - protein, 16 aa, synthetic construct
RSSQSLLHSNVYTYLD

SEQ ID NO: 12 - protein, 7 aa, synthetic construct
LGSNRAS

SEQ ID NO: 13 - protein, 9 aa, synthetic construct
MQALQTPLT

SEQ ID NO: 14 - protein, 5 aa, synthetic construct
SYDIN

SEQ ID NO: 15 - protein, 17 aa, synthetic construct
LINPREDSTSYAQKFQG

SEQ ID NO: 16 - protein, 15 aa, synthetic construct
DLGSIREVLYYGMDV

SEQ ID NO: 17 - protein, 124 aa, synthetic construct
QVQLVQSGAEVKKPGASVKVSCKASGYTFTSYDINWVRQAPGQGLEWVGLINPREDSTSYAQKFQGRVTMTRDTSTSTMYMELSSLRSEDTAVYFCARDLGSIREVLYYGMDVWGQGTTVTVSS

SEQ ID NO: 18 - protein, 112 aa, synthetic construct
DVVMTQSPLSLPVTPGEPASISCRSSQSLLHSNVYTYLDWYLQKPGQSPQLLIYLGSNRASGVPDRFSGSGSGTDFTLKISRVEAEDVGVYYCMQALQTPLTFGQGTRLEIK

SEQ ID NO: 19 - protein, 327 aa, synthetic construct
ASTKGPSVFPLAPCSRSTSESTAALGCLVKDYFPEPVTVSWNSGALTSGVHTFPAVLQSSGLYSLSSVVTVPSSSLGTKTYTCNVDHKPSNTKVDKRVESKYGPPCPPCPAPEFLGGPSVFLFPPKPKDTLYITREPEVTCVVVDVSQEDPEVQFNWYVDGVEVHNAKTKPREEQFNSTYRVVSVLTVLHQDWLNGKEYKCKVSNKGLPSSIEKTISKAKGQPREPQVYTLPPSQEEMTKNQVSLTCLVKGFYPSDIAVEWESNGQPENNYKTTPPVLDSDGSFFLYSRLTVDKSRWQEGNVFSCSVMHEALHNHYTQKSLSLSLGK

SEQ ID NO: 20 - protein, 107 aa, synthetic construct [sequence omitted]

SEQ ID NO: 21 - protein, 451 aa, synthetic construct
QVQLVQSGAEVKKPGASVKVSCKASGYTFTSYDINWVRQAPGQGLEWVGLINPREDSTSYAQKFQGRVTMTRDTSTSTMYMELSSLRSEDTAVYFCARDLGSIREVLYYGMDVWGQGTTVTVSSASTKGPSVFPLAPCSRSTSESTAALGCLVKDYFPEPVTVSWNSGALTSGVHTFPAVLQSSGLYSLSSVVTVPSSSLGTKTYTCNVDHKPSNTKVDKRVESKYGPPCPPCPAPEFLGGPSVFLFPPKPKDTLYITREPEVTCVVVDVSQEDPEVQFNWYVDGVEVHNAKTKPREEQFNSTYRVVSVLTVLHQDWLNGKEYKCKVSNKGLPSSIEKTISKAKGQPREPQVYTLPPSQEEMTKNQVSLTCLVKGFYPSDIAVEWESNGQPENNYKTTPPVLDSDGSFFLYSRLTVDKSRWQEGNVFSCSVMHEALHNHYTQKSLSLSLGK

SEQ ID NO: 22 - protein, 219 aa, synthetic construct
DVVMTQSPLSLPVTPGEPASISCRSSQSLLHSNVYTYLDWYLQKPGQSPQLLIYLGSNRASGVPDRFSGSGSGTDFTLKISRVEAEDVGVYYCMQALQTPLTFGQGTRLEIKRTVAAPSVFIFPPSDEQLKSGTASVVCLLNNFYPREAKVQWKVDNALQSGNSQESVTEQDSKDSTYSLSSTLTLSKADYEKHKVYACEVTHQGLSSPVTKSFNRGEC